European Patent Application EP 4 509 605 A1, published February 19, 2025. Title: Novel lipase. Applicant: 花王株式会社. The sequence listing filed with the application follows.

SEQUENCE LISTING (20 sequences)

SEQ ID NO: 1 - DNA, 876 bp, synthetic construct
  source 1..876: mol_type = other DNA; note = Cedecea sp.-derived sequence
atgtctacatcactgaaatatccgattgtccttgttcatggcctgcttggatttgataaaattggcggaatctacccgtacttttacggaatcaaagaagcgctggaaaaagcaggcgcgaaagtgtatatcgcaacattaagcgcgctgaattctaacgaaatgagaggagaacaattactggaatttgtgcgcaaagtccaggctgaaacaggcgcagcgaaagttaatcttattggccattctcaaggaccgttagcttgcagatatgtggctgccacacatccggatctgatcgcctcagttacaagcgtgaatggcgtcaaccatggatcagaagttgctgatcttgtgagactggcccttaaaccgggacgcttaccggaatcaattgcaaatgcagcgctgagcgcgtttggccaacttttatctgctttagctggagaaccgagactgcctcagtcaggcgtggatgcacttgatgcgttaacaagcgaaggagtcgctgcctttaacaaaaaatatccgcaaggattacctgcagaatggggcggacagggaaaagaactggataacggagtctactactacagctggtctggaattatcgattataacccgctgcatcaaggcatgaataacctggatccgcttcatgttgctatgcttgcctttagcatcctgtttacaaacgaaagatttcagaacgatggcctggtgggacgctattcaagccatcttggcaaagtcattggatctgattattcaatggatcatgttgatgcgatcaatcaactggctggagttgtggccaataacacagatccggtcaaactttatgttgatcatttagcaagactgcaggcgaaaggctta

SEQ ID NO: 2 - protein, 292 aa, Cedecea sp.
MSTSLKYPIVLVHGLLGFDKIGGIYPYFYGIKEALEKAGAKVYIATLSALNSNEMRGEQLLEFVRKVQAETGAAKVNLIGHSQGPLACRYVAATHPDLIASVTSVNGVNHGSEVADLVRLALKPGRLPESIANAALSAFGQLLSALAGEPRLPQSGVDALDALTSEGVAAFNKKYPQGLPAEWGGQGKELDNGVYYYSWSGIIDYNPLHQGMNNLDPLHVAMLAFSILFTNERFQNDGLVGRYSSHLGKVIGSDYSMDHVDAINQLAGVVANNTDPVKLYVDHLARLQAKGL

SEQ ID NO: 3 - DNA, 861 bp, synthetic construct
  source 1..861: mol_type = other DNA; note = Proteus vulgaris-derived sequence
atgagtacgacttatccgattgttttggtacacggactctccggctttgatgacatagtcggctacccttatttttacggaatcgcagacgcactggagaaggacggacataaagtgttcacggcctcgctttcggcttttaacagcaatgaagtccgcggagagcagctttgggaatttgttcaaaaaattctgaaggaaacaaaagcgaagaaagttaacctgatcggccattcacaaggaccgcttgcctgcaggtacgtggcagcaaagcatgcaaaaagcatagcatctgttacatctgtcaacggagtgaatcacggcagtgaaattgcggatttggtgcgccggatcatgagaaaagacagcgtaccagagtacattgctgatgcggtcatgaaagcgatcggtaccatcattagcaccttttccgggaaccgaggaaatccgcaggatgccattgccgcgttagaggctttaactacagaaaatgtgatggaattcaataaaaaatatcctcaaggtcttccagccattcgcggcggcgaaggcaaggaagtggtcaatggtgttcattattattcatttggttcttatattcaaggcctcatcgcgggagaaaaagggaatcttttggatcccacacacgctgcgatgcgtgtattgtcagcgtttttctctgaaagagaaaacgacggcttagtaggcagaacgagcatgcggttaggaaaactgattaaagatgattatgcagaggatcatttagatatggtgaaccaggttgctgggctcgtcgggcgtggggaagatatcattgcaatatatacaaatcatgccaatttcctggcttcaaaaaagcta

SEQ ID NO: 4 - protein, 287 aa, Proteus vulgaris
MSTTYPIVLVHGLSGFDDIVGYPYFYGIADALEKDGHKVFTASLSAFNSNEVRGEQLWEFVQKILKETKAKKVNLIGHSQGPLACRYVAAKHAKSIASVTSVNGVNHGSEIADLVRRIMRKDSVPEYIADAVMKAIGTIISTFSGNRGNPQDAIAALEALTTENVMEFNKKYPQGLPAIRGGEGKEVVNGVHYYSFGSYIQGLIAGEKGNLLDPTHAAMRVLSAFFSERENDGLVGRTSMRLGKLIKDDYAEDHLDMVNQVAGLVGRGEDIIAIYTNHANFLASKKL

SEQ ID NO: 5 - DNA, 870 bp, synthetic construct
  source 1..870: mol_type = other DNA; note = Pseudomonas frederiksbergensis-derived sequence
atgaatatggacgcgtcaacgcaatatccgatagtgcttgttcacggtttgtttggcttcgatacaatcggcggatacccttatttttttgaaatcaaagaagcgcttgaaagggcgggagcaaaagtgtacgctgtcaatattccagcggttaacggcaatgaagagcggggagaaaaactattggagcatgtgaaccgcattcttcgcgaaacaggcgccgccaaggtcaacctgatcggacattcacaaggcccgctggcagcccgatacgtggcagctctgcatccgcaaaaagtagccagtgtcactagtgtgagctgtcccaatcatggatcggaaattgctgatcagcttcataaagcgctgacgcctggcgagctgccagaagcagttgttctggcattattcgccgctgtcggcattttcatctccctaatatccgggcatcctgaaaatccgcaggacgcgcgtgctgcctttgcatcactcacctctgaaggtcttgcggcttttaacaaaaagtatccccagggggttccgaaacattggggtggcgacgggaatgagattgaaaacggagtttattattactcttggtcaggtattgttcagaattttcaatccttacagccactggatccgagccacttaaactgcattgtgctcagtaagctgttttataaagagaaacacgcgaatgacggacttgtcggacaaaacagctctcatttggggaaagtaatcagatctgattatccgatggatcattttgatgctgtaaatcaaatggcagggattacaagctggaatgtctcgcctgtacacctctatttggaacacgcagcaagattaaaggataaaggctta

SEQ ID NO: 6 - protein, 290 aa, Pseudomonas frederiksbergensis
MNMDASTQYPIVLVHGLFGFDTIGGYPYFFEIKEALERAGAKVYAVNIPAVNGNEERGEKLLEHVNRILRETGAAKVNLIGHSQGPLAARYVAALHPQKVASVTSVSCPNHGSEIADQLHKALTPGELPEAVVLALFAAVGIFISLISGHPENPQDARAAFASLTSEGLAAFNKKYPQGVPKHWGGDGNEIENGVYYYSWSGIVQNFQSLQPLDPSHLNCIVLSKLFYKEKHANDGLVGQNSSHLGKVIRSDYPMDHFDAVNQMAGITSWNVSPVHLYLEHAARLKDKGL

SEQ ID NO: 7 - DNA, 882 bp, synthetic construct
  source 1..882: mol_type = other DNA; note = Enterobacillus tribolii-derived sequence
atgaaaaaagcaactacgcttaaatatccgattatcttggtgcacggactttttggttttgacaaaatcgctggcgtttatccttattttttcggtgtaaaagaagctcttgaaaaagcgggggcggaagtgtatgtcgcatcactgtcggcagtaaattcaaacgaagttcgcggtgagcagctcatggactttgtcaatgaggtgctggcaaataccggtgcaaagaaggtgaacttgatcggccactctcaaggcccgcttgcctgccgttacgtggctgcattacgccctgatattgttgcttctgtgacaagcgttcatggcgtcaacttcggcagcgagttagccgatgtggtccgtcaggccttgattccagggaggttgcctgaagcgatagctcatgcggtagtcacaacatttggagatttcttatcgctaatttcaggaaagccgatgcttgcgcaggatgcaaaagccgccttagacgcccttacctcagaaggaatcgcagaatttaatgcgaagtacccgcaagggctgccatctgaatggggaggagaaggcgatgaatatgtaaacggcgtatattattacagctggggcggagttttaaaatacaatatctttgatcagctgttgaacaatctggatcccacacatattgcgatgagtgctctttccattttctttaacaaagagcggggacaaaatgacggcgttgtcggtagatactctatgcatttaggaaaagttatacgatctgattattcaatggatcacctcgacgctgtaaatcaaacggcaggggttgtcacgactagtgtcaatccggtgaagctgtatgttgatcatttgtatcttctgagaagcaaaggcctc

SEQ ID NO: 8 - protein, 294 aa, Enterobacillus tribolii
MKKATTLKYPIILVHGLFGFDKIAGVYPYFFGVKEALEKAGAEVYVASLSAVNSNEVRGEQLMDFVNEVLANTGAKKVNLIGHSQGPLACRYVAALRPDIVASVTSVHGVNFGSELADVVRQALIPGRLPEAIAHAVVTTFGDFLSLISGKPMLAQDAKAALDALTSEGIAEFNAKYPQGLPSEWGGEGDEYVNGVYYYSWGGVLKYNIFDQLLNNLDPTHIAMSALSIFFNKERGQNDGVVGRYSMHLGKVIRSDYSMDHLDAVNQTAGVVTTSVNPVKLYVDHLYLLRSKGL

SEQ ID NO: 9 - DNA, 882 bp, synthetic construct
  source 1..882: mol_type = other DNA; note = Escherichia sp.-derived sequence
atgaagattcagacgcaattaaattaccctgtcgtgcttgtccacggcttgttcggttttgataaaattgcaggggtttatccgtatttttacggcatcaaagatgccttggaagaagctggggccaccgtgttcatcgcttctatttcagcagtaaatgacaatgagcttcggggagagcagctgcttgcatatatcaatgatgtgctgaaaaaaacaggaaaagagaaggttaacctcatcggccattcacaggggcctttggcttgccgctatgtggctgcaacacaccccacattagttgcctctgtcacttctgtaaacggtgtgaatttcggctcagagttcgcggacctcgttagatctgcgctcattccgggtgaaatccctgaagtcattgccaacagtatacttgacgtttttgcgaagctgctgacggccatctccggaaatccggattttccgcaggattcgatagctgcgctggatgcgctaacaacggaaggggtagcaaaatttaacgaaaaatatcctcaaggactcccgattgtacgcggcggtgaaggcaaagaatttgacaacggtgtatattattacagctggagcggcattatagacagcaatatcctgcatcaaggcatgaataactttgatccatctcatattgcgatgctcgcttgtagcatgctgtttgaaaatgaatatcatgaaaacgacggacttgtcggccgttatgcgtcccacttaggaaaggttatcagaagcgattattcgcttgatcatttggatgcaattaatcaaattgcaggagtgttgccacgatacagtgattcaatctccatttaccttgagcatttagagaggttaaaatcaaaaggatta

SEQ ID NO: 10 - protein, 294 aa, Escherichia sp.
MKIQTQLNYPVVLVHGLFGFDKIAGVYPYFYGIKDALEEAGATVFIASISAVNDNELRGEQLLAYINDVLKKTGKEKVNLIGHSQGPLACRYVAATHPTLVASVTSVNGVNFGSEFADLVRSALIPGEIPEVIANSILDVFAKLLTAISGNPDFPQDSIAALDALTTEGVAKFNEKYPQGLPIVRGGEGKEFDNGVYYYSWSGIIDSNILHQGMNNFDPSHIAMLACSMLFENEYHENDGLVGRYASHLGKVIRSDYSLDHLDAINQIAGVLPRYSDSISIYLEHLERLKSKGL

SEQ ID NO: 11 - DNA, 882 bp, synthetic construct
  source 1..882: mol_type = other DNA; note = Yersinia enterocolitica-derived sequence
atgagcacgaacagcactttaaaatacccggttgtgttagttcacggcctgcttggttttgataagatcgccggtgtttatccatatttttacggcgttgaagaacctttgaaaaaagcgggcgcacaggtgtttgtcgcaaccatctccgctacaaactcaaatgaagtaagaggcgaacagcttttgaagtttgtgaaagaagtcatggcaaaaacaggagccaagaaagtgaacttgatcggccacagccaaggcccgctagcttgccgatatgtggcggcgactcatccggagcttattgcatctgtaacgtcagtaaacggggtcaatcacgggagtgagattgctgaccttgtcagatcggctttggtcccaggatcactccccgagcatattgtgaatacaattatgagtgctttcggagtattcgtttctcttttatccggaaaaccgttcctgcctcaggattttatggaaagcatcgacgcgctgaccacagaaaatgtcgcgaaatttaacacgaaatatccgcagggtcttcctgaaacgtgggggggcgaggggaaagaatttgacaatggcgtatattattacagctggggaggtgtccttggctataacccgctcattgaaggcttaaataatctggatccactccatcattctctcgtggccttatcgctgctgttcacaaaagaacgcaaccaaaatgacgggttagtcggtcggtactccatgcatttaggtaaagtcatacgttcagattatcaacttgatcatgttgatgccatcaatcaaacagcaggaatggtttcaaaggatatagatcctgttcaattatttgttaatcagattgaattgctgaagtctaaaggactg

SEQ ID NO: 12 - protein, 294 aa, Yersinia enterocolitica
MSTNSTLKYPVVLVHGLLGFDKIAGVYPYFYGVEEPLKKAGAQVFVATISATNSNEVRGEQLLKFVKEVMAKTGAKKVNLIGHSQGPLACRYVAATHPELIASVTSVNGVNHGSEIADLVRSALVPGSLPEHIVNTIMSAFGVFVSLLSGKPFLPQDFMESIDALTTENVAKFNTKYPQGLPETWGGEGKEFDNGVYYYSWGGVLGYNPLIEGLNNLDPLHHSLVALSLLFTKERNQNDGLVGRYSMHLGKVIRSDYQLDHVDAINQTAGMVSKDIDPVQLFVNQIELLKSKGL

SEQ ID NO: 13 - DNA, 882 bp, synthetic construct
  source 1..882: mol_type = other DNA; note = KAL-A8
atgaaagttcaaacaacattaaaatacccggttgtgctcgttcacggacttttcggctttgacaaaatcgctggtatttatccttatttttatgggattaaggaagcgcttgaagaagcaggtgcaaccgttttcaccgcttcgatttccgctgtcaacagcaatgaagtgagaggggagcagctgctagcttttgtcaaagatgttttgaaaaaaacaggggctgagaaggtaaatttaatcggacattcacaagggccgcttgcctgtcgctatgtagccgcaactcatccggagctggtcgcgagtgtgacgtctgtaaacggcgtgaacttcggttcagaatttgctgatctcgtcagatcggccctgacgcccggaaagctgccggaagccatagcaaatacggtcatgaatgcgtttgcgcagcttttaactgcaatttcaggcaatcctgaattgcctcaggattccattgctgcattggacgctttaacgacagaaggagtagcaaaatttaacgaaaaatatccgcaaggcctgccagcaacatggggcggagaaggcaaggagtttgataacggtgtttattattacagctggtctggaatcattgattcaaatgtgctgaatcagggaatgaacaacttagacccatcccatattgcgatgcttgcctgcagcatgctgtttgataaagaatatcacgaaaatgacggccttgtcggccgttacgcgtctcaccttggaaaagtaataaggtctgattattcactcgatcatcttgatgccatcaatcaaatcgcaggagtgttaccatctgacagtgatgcgattgccatttacgttgagcatatcgcgcggctgaagagcaaaggctta

SEQ ID NO: 14 - protein, 294 aa, synthetic construct
  source 1..294: note = KAL-A8
MKVQTTLKYPVVLVHGLFGFDKIAGIYPYFYGIKEALEEAGATVFTASISAVNSNEVRGEQLLAFVKDVLKKTGAEKVNLIGHSQGPLACRYVAATHPELVASVTSVNGVNFGSEFADLVRSALTPGKLPEAIANTVMNAFAQLLTAISGNPELPQDSIAALDALTTEGVAKFNEKYPQGLPATWGGEGKEFDNGVYYYSWSGIIDSNVLNQGMNNLDPSHIAMLACSMLFDKEYHENDGLVGRYASHLGKVIRSDYSLDHLDAINQIAGVLPSDSDAIAIYVEHIARLKSKGL

SEQ ID NO: 15 - DNA, 879 bp, synthetic construct
  source 1..879: mol_type = other DNA; note = uncultured bacterium-derived sequence
atgtcggcttctagcctgaaatttccgatcgtgctcgttcacggcctgttaggttttgataaaatcggcggaatctatccttatttttacggcattaaagaggcgcttgaaaaagcgggagcgaaggtttatattgcgacactttctgctttgaacagcaatgaacttcgcggagaacagttgttggaatttgtcagaaaagttcaggcagaaacaggcgcggcaaaagtgaatcttattggacactcacaaggcccgctggcatgccgctatgtggcggccactcatccggagctgattgcatctgtcacgtcggtaaacggcgtcaatcatgggagtgaagtggctgatcttgtaagattggctctgacaccgggacgactccctgaatccatagccaatgcagcgatgtcagcattcggacagttactctcggcattggccgggtcaccccgtcttccacagtcaggaattgaagcattagaagctttaacgtctgaaggagttgccgcctttaacaataaatatccgcaaggactgcctgctgaatggggcggtgagggcaaagaattggtaaacggtgtatattattactcttggagcggtgtgattgattataaccctcttcatcagggggcaaacaacttagacccgcttcatgtcgcaatgctggctttctccatcctgtttactaatgagcgttttcaaaatgacgggcttgtcggccggtactcctcacacctaggaaaagtcattgggagtgattacagcatggatcatgttgatgcgatcaatcaattagccggtgttgtcgctaataacaccgacccagttcaattattcgtggagcatgtggcgaggctgaagagcaagggcctc

SEQ ID NO: 16 - protein, 293 aa, unidentified
  source 1..293: note = uncultured bacterium-derived sequence
MSASSLKFPIVLVHGLLGFDKIGGIYPYFYGIKEALEKAGAKVYIATLSALNSNELRGEQLLEFVRKVQAETGAAKVNLIGHSQGPLACRYVAATHPELIASVTSVNGVNHGSEVADLVRLALTPGRLPESIANAAMSAFGQLLSALAGSPRLPQSGIEALEALTSEGVAAFNNKYPQGLPAEWGGEGKELVNGVYYYSWSGVIDYNPLHQGANNLDPLHVAMLAFSILFTNERFQNDGLVGRYSSHLGKVIGSDYSMDHVDAINQLAGVVANNTDPVQLFVEHVARLKSKGL

SEQ ID NO: 17 - DNA, 807 bp, synthetic construct
  source 1..807: mol_type = other DNA; note = Thermomyces lanuginosus-derived sequence
gaagtgagccaagatttatttaaccagtttaacctgtttgcgcaatattctgcagcggcttattgcggaaaaaataacgatgccccggcaggaacaaatatcacatgcacaggcaacgcttgtccggaagttgaaaaagcggatgctacatttctttactcatttgaagatagcggcgtgggagatgtcacaggctttctggcccttgataacacaaacaaactgatcgtgctgtcatttagaggaagccgctctatcgaaaactggatcggcaaccttaactttgatctgaaagaaatcaacgatatctgctcaggctgtagaggacatgatggctttacatcaagctggagaagcgtcgcggatacattacgccagaaagttgaagatgctgtgagagaacatccggattatcgcgttgtgtttacaggacattctctgggcggagcccttgcaacagttgctggagctgatctgagaggcaacggatacgatatcgatgtcttttcatacggagctccgagagttggcaaccgcgcctttgcagaatttcttacagtgcaaacaggcggaacactgtaccgcatcacacatacaaacgatattgtcccgagactgccgccgcgcgaatttggatattctcattcttcaccggaatattggatcaaatcaggcacacttgtcccggttacacgcaacgatatcgttaaaatcgaaggaatcgatgccacaggcggaaataaccagccgaacatcccggatattccggcacatttatggtattttggactgattggcacatgtctt

SEQ ID NO: 18 - protein, 269 aa, Thermomyces lanuginosus [sequence omitted]

SEQ ID NO: 19 - DNA, 99 bp, synthetic construct
  source 1..99: mol_type = other DNA; note = Bacillus subtilis-derived sequence
atgtttgcaaaacgattcaaaacctctttactgccgttattcgctggatttttattgctgtttcatttggttctggcaggaccggcggctgcgagtgct

SEQ ID NO: 20 - protein, 33 aa, Bacillus subtilis
MFAKRFKTSLLPLFAGFLLLFHLVLAGPAAASA